European Patent Application EP 4 660 200 A1, published December 10, 2025. Title: Silent mutations. Applicant: MU Bioteknik Aktiebolag. The sequence listing filed with the application follows.

SEQUENCE LISTING (11 sequences)

SEQ ID NO: 1 - protein, 58 aa, synthetic construct [sequence omitted]

SEQ ID NO: 2 - protein, 58 aa, synthetic construct [sequence omitted]

SEQ ID NO: 3 - protein, 58 aa, synthetic construct [sequence omitted]

SEQ ID NO: 4 - protein, 55 aa, synthetic construct
AKFDKEQQNAFYEILHLPNLTEEQRNAFIQSLKDDPSQSANLLAEAKKLNDAQAP

SEQ ID NO: 5 - protein, 58 aa, synthetic construct
ADAKFDKEQQNAFYEILHLPNLTEEQRNGFIQSLKDDPSQSANLLAEAKKLNDAQAPK

SEQ ID NO: 6 - protein, 55 aa, synthetic construct
AKFDKEQQNAFYEILHLPNLTEEQRNGFIQSLKDDPSQSANLLAEAKKLNDAQAP

SEQ ID NO: 7 - DNA, 921 bp, synthetic construct
  source 1..921: mol_type = other DNA
gcgcaacacgatgaagctgttgatgcaaaattcgataaagaacaacaaaatgctttctatgaaatcttacatttacctaacttaacggaagaacaacgcaatgccttcatccaaagcctaaaagatgacccaagccaaagcgctaaccttttagcagaagctaaaaagctaaatgatgctcaagcaccaaaagttgatgcaaaattcgataaagaacaacaaaatgctttctatgaaatcttacatttacctaacttaacggaagaacaacgcaatgccttcatccaaagcctaaaagatgacccaagccaaagcgctaaccttttagcagaagctaaaaagctaaatgatgctcaagcaccaaaagttgatgcaaaattcgataaagaacaacaaaatgctttctatgaaatcttacatttacctaacttaacggaagaacaacgcaatgccttcatccaaagcctaaaagatgacccaagccaaagcgctaaccttttagcagaagctaaaaagctaaatgatgctcaagcaccaaaagttgatgcaaaattcgataaagaacaacaaaatgctttctatgaaatcttacatttacctaacttaacggaagaacaacgcaatgccttcatccaaagcctaaaagatgacccaagccaaagcgctaaccttttagcagaagctaaaaagctaaatgatgctcaagcaccaaaagttgatgcaaaattcgataaagaacaacaaaatgctttctatgaaatcttacatttacctaacttaacggaagaacaacgcaatgccttcatccaaagcctaaaagatgacccaagccaaagcgctaaccttttagcagaagctaaaaagctaaatgatgctcaagcaccaaaaggtggcggcggttccggcggtggcggtagctgt

SEQ ID NO: 8 - DNA, 921 bp, synthetic construct
  source 1..921: mol_type = other DNA
gcgcaacacgatgaagctgttgatgcaaaattcgataaagagcaacaaaatgctttctatgaaatcttacacttacctaacttaacggaagaacaacgcaacgccttcatccaaagcctaaaagatgacccgagccaaagcgctaaccttttagcagaagcaaaaaagctaaatgatgctcaagcaccaaaagttgatgcaaaattcgataaagaacagcaaaatgctttctatgaaatcttacatctgcctaacttaacggaagaacaacgcaatgctttcatccaaagcctaaaagatgacccatctcaaagcgctaaccttttagcagaagctaagaagctaaatgatgctcaagcaccaaaagttgatgcaaaattcgataaagaacaacagaatgctttctatgaaatcttacatttaccgaacttaacggaagaacaacgcaatgcctttatccaaagcctaaaagatgacccaagccagagcgctaaccttttagcagaagctaaaaaactaaatgatgctcaagcaccaaaagttgatgcaaaattcgataaagaacaacaaaacgctttctatgaaatcttacatttacctaatttaacggaagaacaacgcaatgccttcattcaaagcctaaaagatgacccaagccaaagtgctaaccttttagcagaagctaaaaagctgaatgatgctcaagcaccaaaagttgatgcaaaattcgataaagaacaacaaaatgccttctatgaaatcttacatttacctaacctgacggaagaacaacgcaatgccttcatccagagcctaaaagatgacccaagccaaagcgccaaccttttagcagaagctaaaaagctaaacgatgctcaagcaccaaaaggtggcggcggttccggcggtggcggtagctgt

SEQ ID NO: 9 - DNA, 921 bp, synthetic construct
  source 1..921: mol_type = other DNA
gcgcaacacgatgaagctgttgatgctaaattcgataaagagcaacaaaatgctttttatgaaatcttacacttacctaacttaactgaagaacaacgcaacgccttcatccaatctctaaaagatgacccgagccaaagcgctaatcttttagcagaagcaaaaaagctaaatgacgctcaagcaccaaaagttgatgcaaagttcgataaagaacagcaaaatgctttctacgaaatcttacatctgcctaacttaacggaggaacaacgcaatgctttcatccaaagcttaaaagatgacccatctcaaagcgctaacttgttagcagaagctaagaagctaaatgatgcccaagcaccaaaagttgatgcaaaatttgataaagaacaacagaatgctttctatgagatcttacatttaccgaacttaacggaagagcaacgcaatgcctttatccaaagcctaaaggatgacccaagccagagcgctaaccttctggcagaagctaaaaaactaaatgatgctcaggcaccaaaagttgatgcaaaattcgacaaagaacaacaaaacgctttctatgaaattttacatttacctaatttaacggaagaacagcgcaatgccttcattcaaagcctaaaagacgacccaagccaaagtgctaaccttttagctgaagctaaaaagctgaatgatgctcaagccccaaaagttgatgcaaaattcgataaggaacaacaaaatgccttctatgaaatcttgcatttacctaacctgacggaagaacaacgtaatgccttcatccagagcctaaaagatgatccaagccaaagcgccaaccttttagcagaggctaaaaagctaaacgatgctcaagcaccgaaaggtggcggcggttccggcggtggcggtagctgt

SEQ ID NO: 10 - protein, 6 aa, synthetic construct
AQHDEA

SEQ ID NO: 11 - protein, 11 aa, synthetic construct
GGGGSGGGGSC